European Patent Application EP 4 549 453 A1, published May 7, 2025. Title: 一种提高香兰素产量的重组拟无枝酸菌、其构建方法及应用. Applicant: 陕西海斯夫生物工程有限公司. The sequence listing filed with the application follows.

SEQUENCE LISTING (8 sequences)

SEQ ID NO: 1 - DNA, 1413 bp, Amycolatopsis sp.
  source 1..1413: mol_type = other DNA
atggtggatcagcgggcggtcctgccgccccggctggccgcgtcctggcagcgcagcaggcagtacggggtgtcaccggagacggtgcggccggcgttcaccggcaccgtcgaccacgattcgctgttcttcgagtgcggccaggaggtgctctccggcctgcacaccaccctggccaacgaaccggtcagcctgatgctcaccgacagtgacggcctggtgctgagccggctgtgcgacgacagcaccatcctccgttcgctggaccgcgtccacctggcgccgggcttctcctacgcggagcgcgacgccggcaccaacgggctcggcctcgcgctggccgaccgcgccccgtcgctggtgtccgccgaggagcactactgcacgggcctgtggggctacacctgcgccgccgcgccggtgctggagccgggcacgaaccggctcatcggcagcgtcaacctgaccacgtggtcgaagtcgtcgaaggagctgctgctcgcgctggcccaggccgcggcgggcaacacggcggcgctgatgctcgcccggtcgcacggccacctcgcgccgccgggcccgcgtggcgaggtgttccgcgtctactccgaccggctgcccgacgtcgcggcgaacctgtccaccgcctggtccgacgcgctcgccgaggcccgcacagcaatggagcacggccgcgtggtgtgcgtgaccggtgagccgggcagcgggaaggccgcgctggcgtcgatggcccgccggtcggtgcgcccgcgggaacgcgtcctcaacgcccggccgcccgcgccgcaggacgcggcgtcgtggctggcgctgtggacgccggaggtcggcaaggccgacacgtgcgtgatcctctccggcgccgacgcgctgcccgcctacgccgcggaggagctggccgcgctgttcgccgcggcgcgcggcgggttcgtgatgacggccgcggaccacgcgggcgtgccggacgcgctgcgggccctggtcgacgcggtcgtcgaggtgccggcgctgcggtaccggccggacgacgtcctcccgctggccgggcacttcgcgcgggagagccgcggccgcccggtcaccttcacgccggccgcgtcgcgggcgctgaccgcctacccgtggccgggcaacgtccgccagctccggcaggtggtgcgcgaggcggtggcgcgggctgatgtcgtggacacccggcacctgccgccggaggtgttcaccagccccggccgccgcctgacgcggatggaggccgtggagcgcgacgaaatcgtgcgctgcctgaccaaaccgggcacgacggccgcgcaggtggcgtcgatgctgggcatgagccgcgccacggtgtaccgcaagatcgcccagtacgggatcaaggtgccgcgccggtag

SEQ ID NO: 2 - DNA, 954 bp, Amycolatopsis sp.
  source 1..954: mol_type = other DNA
gtgatcgggctcgggttgatcggcggctcggtgctgcgcgcggccgcggcggtggggcgcgaggtgtggggcgcgacgacttcggcggccgacgccgaggcggcggccgccgacgggttcgacgcctcgaccgacgtggaagccgcgctgcggcgggccgccgaccgggacgcgctggtggtgctggccgtgccgctgaccgccgtcgaggaggtgctgcggacggtcgacgtgtgcgcgccgtcgtgcctgctcaccgacgtgaccagcgtgaagacgggtgtgctgacggccgcgcgggcgttcgcgccgaacgcccgatatgtcggcgggcacccgatggcgggcaccgccgagtccggctggcgggccggcaacgccgcgctgttcggcggcgcggcgtgggtggtgtgcgtcgaggacgacaccgatctcggcgcgtgggccgaggtggcccggctggcgatcgacctcggctcgcacgtggttccgctgaccgcggccacgcacgacgaggcggtcgcccggatctcccacctgccgcacctgctggccgcggttctcgcggccgtgggggcggacggcgggccggtcgcgatggcgctggccgccggctcctacaccgacggcacccgcgtggccgccacccggccggcgctggtgcgcgcgatgaccgagggcaaccgcgaagcgctgctgccggtgatcgacgaagccctcggccggctgggcgccctgcgcgggtcgctggcctcgaccggcggcctcgccgtcagcatcgactcgggtcaccagggcgcgcaagcgcttgcggccgccaggcaggccacgctgtcgggcgtccgcgtcgctctgggcgcgccggacgcccgggacggcctgcgtgcgctcggcgagcgcggcggccgcatcacttccctcaccgaggacaccgccatcggcgaggtgccgtaa

SEQ ID NO: 3 - DNA, 1101 bp, Amycolatopsis sp.
  source 1..1101: mol_type = other DNA
atgtctcccagcgcctcgacactcagcgcaggccccgcggacgtcaccgaaggcctcgacaaccagcgcacgctcggcgtcagcccgctgatctcccccgccctgctgcggcaggagctgccggtggacgcggcgatcgccaagaccgtcgcgcagggccggtcgtcggccgtcgacatcctgggcggcgacgacgaccgcctcatcgtggtcgtcggcccgtgctcggtgcacgaccccgcggccgccctcgactacgcccaccggctggccgagcacgccgccggtctgcgcgacgagctgcacgtgatcatgcgggtgtacttcgagaagccgcgcaccacgctgggctggaagggcctcatcaacgacccggacctggacggcagctacgccgtcaacaagggcctgcggatggcgcgcaagctgctgctggacatctccgcgctggggctgccggtcgggtgcgagttcctggacccgatcacgccgcagttcatcgccgacaccgtgagctggggatcgatcggcgcgcggaccgcggcgagccaggtgcaccgccagctgtgcagcgcgctgtccatgccggtggggatcaagaactccaccgagggcgacgtgcaggtggcggtggacgcgacccgcgccgcggcggcgagccacgtgttcgcgggcatcaacaacgacggcctggccgcgctgttcaccaccgcgggcaaccccgactgccacgtcatcctgcgcggcggttccgcgggcccgaactacgacgccgcgacggtggccgacacgctcgcgcggcaggcgaaggccgggctgccggagcgggtgatcatcgacgcgagccacggcaacagcggcaaggaccacgtccgccagggcgtcgtggccggggagatcgcggaccggatcgccgccggcgagcgcgggatcgccgggatcatgctggagagcttcctcgaggccgggcggcaggatctcgtgctggggcgcgccgacgagctgacatacgggcagtcgatcaccgatgcgtgcctggattggcgcagcacgggggagctgttggatcggttggcttcggctgtggctgctcggcggtag

SEQ ID NO: 4 - DNA, 1425 bp, Amycolatopsis sp.
  source 1..1425: mol_type = other DNA
gtgagccgacgcgcgaagatcgtttgtactatgggccccgcgaccgccaccgcggacaaggtgcgagcccttgtcgacgccgggatggacgtggcgcggctgaacttcagccacggcagccacggcgaccacaagcaggtgtacgacctgatccgggaggccgcggccgaaaccgggcgcgcggtcggcatcctcgccgacctgcagggcccgaagatccggctcggcaccttcgcgggcggcccggtcgaatggcgcaccggtgacgtcgtgcgcatcaccgtggaggacgtcgccggcacccacgaccgggtctcgaccacctacaagggcctggccaaggacgccaagccgggcgaccgcctgctcgtcgacgacggcaaggtgggcctggtcgtcaagggcgtcgagggcccggacgtcgtgtgcgaggtcaccgagggcggcccggtcagcaacaacaagggcgtctcgctgcccggcatggacgtctccgtgcccgccctgtccgacaaggacatcgaggacctggagttcgcgctcgaactgggcgccgacttcatcgcgctgtccttcgtccgctcgcccgccgacatcgacctggtccaccaggtgatggaccgcgtcggcaagggccgccgcccggtcatcgccaagctggagaagcccgaggcggtctacaacctggaagccatcgtgctggccttcgacggcgtcatggtcgcccgcggcgacctgggcgtcgagttgccgctggagcaggtgccgctggtccagaagcgcgccatccagatcgcccgcgagaacgccaagccggtcatcgtcgcgacccagatgctcgactcgatgatcaacaactcgcgcccgacccgcgccgaggcctccgacgtggccaacgcggtgctcgacggcgcggacgcggtcatgctgtccggcgagaccagcgtgggccgctacccgatcgagaccgtgcagacaatgtcccggatcgtggaggccgtcgaggccgacaccccggccgtgccgccgctgtcgcacgtgccgcgcaccaagcggggcgtcatctcctacgcggcgaaggacatcggcgagcggctcaacgccaaggcgctggtcgcgttcacgcagtccggcgacacggtccgccgcctcgcccggctgcacacgcggctgccgctgctggcgttcacgccggaggagagcgtgcgcagccagctggcgctgacctggggcacccacaccgagctggtgccgtcggtggactcgaccgaccgcatgatcaagcaggtcgaccgcgcgatgctggagacgggccgttaccaggccggcgacctggtcgtcatcgtggccggctccccgccgggcaccgtcgggtcgaccaacctgatccgcgtgcacaagctcggtgaggacgaccacgcctga

SEQ ID NO: 5 - DNA, 2244 bp, Amycolatopsis sp.
  source 1..2244: mol_type = other DNA
atgactttcgtacgggagctgtccgcgatccgggccgacgacgacctttcggccggcggcaagggcgcgaacctgggtgagctcaccgcggcgggattcccggtgccgcgcgggttcgtcgtgctgcgcgagggctactgggcgaccaccgagtacgacggcgtccgtgacgagctcgcccacctgcacgccgaggcgctcggcctggccgacgaccccgagcggctcgccgagcactgcgaccgcatgcgggacttggtgcgcaaggccaccctcgacccgcgggtccgcgccgaggtggtcgccgcctacgcgcagctggggccggacgccgtggtcgcggtgcggtcgtcggcgaccggggaggacggcgcggacgcctccttcgccgggatgaacgccagcttcaccaacgtcgtcggcgagcacgcgctgctggagcggctcaccgactgctgggcctcgctgttttccccgcgtgtggtcgcctaccgggcaggccgcgggttcaccggcgagccggcgatcgcggtcgtggtgcaggagatggtccgggccgagcgcgccggtgtggcgttcaccgccgacccgcgcaccggcgaccggggagtggtcgtggtcgaggcggtgttcggccagggcgagacgctggtgtcgggcgcggtgtccccggacacctacgtcgtcggcaaggacgacctgaaggtgcgcgaggtgcgcatcggcgacaagacccacaagatcgtccacggccccgacggcgacactcgcgtcgagctgtccgcgagcgccgcgcaccagcgcgtgctcggcgacgtcacggtggtcgggctggcccgcctcgcccggcgcgtggaggagcactacgggcggccgcaggacctggagtgggcggtggacggcgaccggacctggctggtccagacgcggcccatcaccacgctgggcccggagccgaagcccgccgggcaggtgctgctgcgcggtctggccgcgtcgcccggccgggcgggtggcgcggtgcgcgtgctgacccggcccgaccagggcaaggccctgcgcagcggggagatcctcgtcgcgccgatgacgaacccggactgggtgccgacactgcgccgcgcggcggcgatcgtcaccgacggcggcgggatgacctgccacgccgcgatcgtggcccgcgagctgggcgtcccatgcgtcgtcggcgcgggcggcgcgacgacgctgctgaccgacggcgaggaggtgaccgtcgacggcagcaccggggaggtccgcagcggcatcaccgccgcgcccgcccgcacggagcccgtcgcggcccccgcggtggccgccgagcccctcgccacccgcctgtacgtcaacctcgcgatcgccgaccaggccgagcgcgtcgccgcgctccccgtcgacggggtcggcctgctgcgcgcggagttcctgctcaccagtgcgctcggcggacgccacccccgggacctgctggcccgcggcgagggcgagtcgttcgtgacagccatgagcgagtcgctgctgaccatcacccgcgcgttcggcgcccgcccggtcgtctaccgggcaaccgacctgcgcagcaacgagttccgcggcctgaccggcggggagcgctacgagcccgccgagcacaacccgatgatcggctaccgcggctgcttccgctacgtgcgcgagccggacctgttcgacctcgaactgcgggcgctggcgcgggtgcgggaggagaccccgaacctgcacctgatgatcccgttcgtgcgcacgaagtgggagctggaggagtgcctgcgcctggtcgacgccagcccgctcgggcgctcccgcggtctgcgccggtgggtgatggccgaggtgccgtcggtggtgcactggctccccgagtacgtgggcctcggcatcgacggtgtctccatcggcagcaacgacctgacgcagctggtgctcggcgtggaccgcgattcgcgggagtgcgccgagctgttcgacgaatccgacccggcggtgctggacgcgatcgggcggatcgtgacgacggcccggtcgctgggcatcacgtcgtcgctgtgcgggcaggcgccgtccaaccggcccgagttcgccgaccacctggtgcggctgggcatcacgtcgatctcggtcaacccggacgccgtgcccgccgcccggaccgcgatcgcctccgccgagcggcgggtgctgctggagcgcgcccgctcctga

SEQ ID NO: 6 - DNA, 1800 bp, Amycolatopsis sp.
  source 1..1800: mol_type = other DNA
gtggaccacgaccggggcggcgcggtgctcgacgacgtcaagctggcgcgcacccggttgcggttcctgacggccgaagcggtcgagcccgggcaggtccgcgaggcgatcctcgcgtcctggtggcgctcccgcgagttccaggtgcccgccgaccgcatcgacctgccctacagcggcgaccagaacctggacacgccgctgatccgcggcgcgcaaccggtgctggaacggctgggcgaccagctcgacggccagccgatcagcatgatcctcaccgaccagtccggcgtcgtgctcacgcagcgcaccggcgaccacgacctgcaccggcacctgcagagcgtggagctggcgcccgggttcagctatggcgagaagttcgtcggcaccaacgggatcggcaccgcgctcgccgacgggcggccgacgcaggtgttcgggcacgagcactacgcggagaacctggagaacctggcgtgcgcgggcgtgccgatccagcacccgatctccggcaagacgatcggcgccgtggacctgacctgctggcgcaaggacgccggcgggctgctcgtcgcgctcgccaggtcgaccgccgagcagatccggcaggcgctgctcacccacagcaccatgcgcgagctggtgctgttccagacctacctgcaggcctgccgccgcaccaccgggatcgtgatcgcgttcaacgacgacgtggtgatgatgaacgacgccgcccgccagctcctcgacccggtcgaccagtcgctcgtgctcgggcacgccaagcaggcgctgtccgcggcccggcgcgccaccgagacgatcgtgctgtccagcggcggcaaggtgcggatgtactgccgtcgcgtggcgggcgagcggagcggcgagatcgccggcggggtgctgtcggtgcagctggtcgacaccgacgacgggggcgcgggcgtcacgctgcccgccgtgccgatgttcctgcccggcgtggccgggtcggcgccgacgtggtcgcgcagctgccacgccgtcgacagcagcttcgtccgcggcgagtggctggtgctggcaggcgagcccggggtcgggaagcacacgctggcgcagggcgtgcaccggcggcgcaacccggccgggcggctgcacacgctcgacgcggccgaggccggaccgggctgggccggggacgtgcggcacgagctgctcgacgacccggtggacacgctggtgatccggcatgccgaccggctgggcgacgaggacgtgcgcgcgctggtcgccgtgctgcggcaggtgccgcggccggacgggccgtgggtggcgctgacgctgacgccggaggccgagagcagcccgcggctggcggagctgctcgcgttcttcccgcggacggtcggggtgccgtcgctgcggcggcacgtggaggacctggccgagctggtgccgctgttcctcagcaagctgtcgcacggcgggcagatcacgtgctcaccggaggcgatgcacctgttgatgcgggcgtcatggccgggcaacacggcgcagctgcaccaggtgctgcgggaaatcacccagcggcgccgcactgggaccatccggccgaacgacctgccggccgagtaccacaccatcacgcggcgtccgctgaaccggttcgaggccgtcgaacgcgacgcgatcgtgcgcagcctggaggacgcgggcggcaacaaggcccgcgcggcgcaactgctgggcatctcccgcgcgacgatctaccggaagatccacgagtacgggatcgtcacgccggtgcactga

SEQ ID NO: 7 - DNA, 1683 bp, Amycolatopsis sp.
  source 1..1683: mol_type = other DNA
atgggcgtcgacgggttcgaggcgaccgccgtggccggcgagctgccgagcgcggcggaagccgagatccgggattcgtggcgccgctcctggcggtccggggtacggcccgacctgccactcgagcggctcgacgcggtggacgtcgaccagcgaagccgcctgttgcgggccgcgttgcccgtgctcgaccaggttgccgccgaactcggcgagacggcctacttcaccgtcctggccgacagcgccgcccggatcgtccaccggggacgcatcagttcgcgcacggccgacatcctcgacgacaccggggtcgtcctgggcaggcggttcaccgaggacacgaccggcaccaacgccatcgccacaccgtttgagcttcgccggggcgtggcggtgcgtggcggcgagcacttcgcccggtcgctgcgtggctacagctgctacggctacccgatagtgcaccccgcgacgcggcggctcgaaggcgtcctcgacctcgccgggccggcaggtggggagaacccgctgttcggcccgttcttgcggcaggccgtccggcagatcgaaagcgccttgctggccgactcccgtgattccgaacgacgtctcctcgacgcgttcaaccgggccgtggccaggcgtggcgaacgggcggttctggcgctcggcgacgacggcgtggtgctcgccaaccagcaggcgctggaccacttcgacgccctcgaccacgagcgactccgggagctggcacatgggccgcggtgggacgggaagtcccgcgaggtggtcttcgagacggcgcacgggatgcggttgcgactgacgctcgaacccgtgggcgggcacggaaacgtgctgatccggttcacccccgcctaccggtcgcatcccgtggttccccggaggcaggccaccgcccgcgacgtcctcgaccgggaactggcgagataccgcgcggcgcgcctggcgaccttcatcgcgggagaagccggaaccgggcgcacccggacggcgcacagcctggcatccggtaccggcgccgaggtggtgaccgtcggcggccatgaaccggtcgaggggtccacctggctccaccgggtccgcagcgccgccgcctccggcgcgctggtcgtcgtcgagggtgtcgaactgctcgacgacacggtggtgcgggcgctcggggagtgcgtcgcgcaggggatctggacggcgatcacggggccgccggtggatcggctcggtccacggcaccggcacctcgccttccggtgccccggacgtctggaactgccgcccctgcgcgagcggcgcgcggacatcccggcgctggcccgggcgatgctcgccgaggcgacgagcgggtccgcccggttcacgcccgccgccctggcgtgcctcgcggagctggactggcccggcaacctgcgggagctcgatcacgtcgtacgccgggtcgccgccaaacgcagcacgggcgacatcgtcgccggtgacctgccgcgggaataccgcggcgcccccgccaaggctcgccttactccctgggaacggtccgagcacgacgcgatcctggccgctctcgaacgcaaccaggggaacaagacccgcgcggccgaggacctcggcatcagccgcggaacgctgtacaaccggatcagggtgctgcggatccgcgtgtga

SEQ ID NO: 8 - DNA, 1392 bp, Amycolatopsis sp.
  source 1..1392: mol_type = other DNA
gtgaactggaccgtggacgtgcccgtcgacacccttcccgagctgccgcccctgccgccggaactgcgtgcccggctggacgacgccctgtcccgccccgccgcccagcagccggagtggcccgacgccgacgcggtcggccgggtccgccacctgctcgaggccgtgccgcccatcaccgtgcccgccgagatcgaccggctccaggaccgcctcgccatggtcgcccgcggcgaggccttcctgctccagggcggcgactgcgccgagacgttcgagtccaacaccgagccgcacatccgcgccaacctgcgcacgctcctgcagatggccgtcgtcctcacctacggcgccagcctgcccgtcgtgaaggtcgggcgcatcgcgggccagtacgccaaaccgcgctccaacagcaccgacgcgctcggcctgcccgtctaccgcggcgacatcgtcaactcgctcgtcgccaagcccgagctgcgcgtccccgacccgggccgcatgatccgcgcctacgccaactccggcgcggcgatgaacctggtccgcgccctcaccggcgccggcatggccgacctcgcccaggtgcacgactggaacaaggacttcgtccgcacctcgcccgcgggcgagcgctacgaggcgctggccggcgaaatcgaccgcggcctgcggttcatgtccgcctgcggcgtcagcgacacctcgctgcactccaccgagatcttcgccagccacgaggccctgctgctcgactacgagcgcgccatgctgcggatggacaacgccaacgcggccaacccgaagctgtacaacctctcgtcccacttcctgtggatcggcgagcgcacccgccagctcgacggcgcccacatcgccctcgccgaactgctggccaaccccatcggcgtgaagatcggcccgaccaccacgcccgagcaggccgtggagtacgtcgagcgcctcgacccgcgcaaccagcccggccgcgtcaccctcatctcccgcatgggcaacggcaaggtccgcgacgtcctgcccgccatcgtggagaaggtcgaggccaccggccacaaggtgatctggcagtgcgacccgatgcacggcaacacgcacgagtcgtccagcggctacaagacccgccacttcgaccgcatcatcgacgaggtccagggcttcttcgaggtgcaccacaagctcggcagctaccccggcggcatccacatcgagctcaccggcgaggacgtcaccgagtgcctcggcggggcgcaggagatctccgactccgatctggccgggcggtacgagacggcctgcgatccgcggctgaacacgcagcagtcgctggagttggcgttcctggtggcggagatgttgcggggttga